European Patent Application EP 4 814 124 A1, published September 30, 2026. Title: がんの遺伝子治療薬. Applicant: 国立大学法人神戸大学. The sequence listing filed with the application follows.

SEQUENCE LISTING (51 sequences)

SEQ ID NO: 1 - DNA, 735 bp, Homo sapiens
  source 1..735: mol_type = other DNA
atggacaagttttggtggcacgcagcctggggactctgcctcgtgccgctgagcctggcgcagatcgatttgaatataacctgccgctttgcaggtgtattccacgtggagaaaaatggtcgctacagcatctctcggacggaggccgctgacctctgcaaggctttcaatagcaccttgcccacaatggcccagatggagaaagctctgagcatcggatttgagacctgcaggtatgggttcatagaagggcacgtggtgattccccggatccaccccaactccatctgtgcagcaaacaacacaggggtgtacatcctcacatccaacacctcccagtatgacacatattgcttcaatgcttcagctccacctgaagaagattgtacatcagtcacagacctgcccaatgcctttgatggaccaattaccataactattgttaaccgtgatggcacccgctatgtccagaaaggagaatacagaacgaatcctgaagacatctaccccagcaaccctactgatgatgacgtgagcagcggctcctccagtgaaaggagcagcacttcaggaggttacatcttttacaccttttctactgtacaccccatcccagacgaagacagtccctggatcaccgacagcacagacagaatccctgctaccagacactcacatgggagtcaagaaggtggagcaaacacaacctctggtcctataaggacaccccaaatt

SEQ ID NO: 2 - DNA, 1029 bp, Homo sapiens
  source 1..1029: mol_type = other DNA
atcctggactacagcttcgggggtggggccgggcgcgacatccccccgccgctgatcgaggaggcgtgcgagctgcccgagtgccaggaggacgcgggcaacaaggtctgcagcctgcagtgcaacaaccacgcgtgcggctgggacggcggtgactgctccctcaacttcaatgacccctggaagaactgcacgcagtctctgcagtgctggaagtacttcagtgacggccactgtgacagccagtgcaactcagccggctgcctcttcgacggctttgactgccagcgtgcggaaggccagtgcaaccccctgtacgaccagtactgcaaggaccacttcagcgacgggcactgcgaccagggctgcaacagcgcggagtgcgagtgggacgggctggactgtgcggagcatgtacccgagaggctggcggccggcacgctggtggtggtggtgctgatgccgccggagcagctgcgcaacagctccttccacttcctgcgggagctcagccgcgtgctgcacaccaacgtggtcttcaagcgtgacgcacacggccagcagatgatcttcccctactacggccgcgaggaggagctgcgcaagcaccccatcaagcgtgccgccgagggctgggccgcacctgacgccctgctgggccaggtgaaggcctcgctgctccctggtggcagcgagggtgggcggcggcggagggagctggaccccatggacgtccgcggctccatcgtctacctggagattgacaaccggcagtgtgtgcaggcctcctcgcagtgcttccagagtgccaccgacgtggccgcattcctgggagcgctcgcctcgctgggcagcctcaacatcccctacaagatcgaggccgtgcagagtgagaccgtggagccgcccccgccggcgcagctgcacttcatgtacgtggcggcggccgcctttgtgcttctgttcttcgtgggctgcggggtgctgctgtcccgcaagcgccggcggcagcatggccagctctggttc

SEQ ID NO: 3 - DNA, 1092 bp, Homo sapiens
  source 1..1092: mol_type = other DNA
atggcgctggggctgcagcgcgcaaggtcgaccacggagctgcgcaaggaaaagtcccgggatgcggcccgcagccggcgcagccaggagaccgaggtgctgtaccagctggctcacacgctgcccttcgcccgcggcgtcagcgcccacctggacaaggcctctatcatgcgcctcaccatcagctacctgcgcatgcaccgcctctgcgccgcaggggagtggaaccaggtgggagcagggggagaaccactggatgcctgctacctgaaggccctggagggcttcgtcatggtgctcaccgccgagggagacatggcttacctgtcggagaatgtcagcaaacacctgggcctcagtcagctggagctcattggacacagcatctttgatttcatccacccctgtgaccaagaggagcttcaggacgccctgaccccccagcagaccctgtccaggaggaaggtggaggcccccacggagcggtgcttctccttgcgcatgaagagtacgctcaccagccgcgggcgcaccctcaacctcaaggcggccacctggaaggtgctgaactgctctggacatatgagggcctacaagccacctgcgcagacttctccagctgggagccctgactcagagcccccgctgcagtgcctggtgctcatctgcgaagccatcccccacccaggcagcctggagcccccactgggccgaggggccttcctcagccgccacagcctggacatgaagttcacctactgtgacgacaggattgcagaagtggctggctatagtcccgatgacctgatcggctgttccgcctacgagtacatccacgcgctggactccgacgcggtcagcaagagcatccacacctgtatgtatcccatttccccaggtgcgaagccagctgccacatggcccccagctgacaccaggaccccccagctccccataccccaggatgcactgcctccccacctcaacaccagctccctgctccccaagccccaaggaactgtctccttccttgccccctcatacccagtccccagatctttctctccccatttgcccccttggtggccctga

SEQ ID NO: 4 - DNA, 1567 bp, Homo sapiens
  source 1..1567: mol_type = other DNA
ttgaggtacctggtgtagttttatttcaggttttatgctgtcattttcctgtaatgctaaggacttaggacataactgaattttctattttccacttcttttctggtgtgtgtgtatatatatatgtatatatacacacacacatgtacatatatatattttttagtatctcaccctcacatgctcctccctgagcactacccatgatagatgttaaacaaaagcaaagatgaaattccaactgtcaaaatctcccttccatctaattaattcctcatccaactatgttccaaaacgagaatagaaaattagccccaataagcccaggcaactgaaaagtaaatgctatgttgtactttgatccatggtcacaactcataatcttggaaaagtggacagaaaagacaaaagagtgaactttaaaactcgaatttattttaccagtatctcctatgaagggctagtaaccaaaataatccacgcatcagggagagaaatgccttaaggcatacgttttggacatttagcgtccctgcaaattctggccatcgccgcttcctttgtccatcagaaggcaggaaactttatattggtgacccgtggagctcacattaactatttacagggtaactgcttaggaccagtattatgaggagaatttacctttcccccctctctttccaagaaacaaggagggggtgaaggtacggagaacagtatttcttctgttgaaagcaacttagctacaaagataaattacagctatgtacactgaaggtagctatttcattccacaaaataagagttttttaaaaagctatgtatgtatgtgctgcatatagagcagatatacagcctattaagcgtcgtcactaaaacataaaacatgtcagcctttcttaaccttactcgccccagtctgtcccgacgtgacttcctcgaccctctaaagacgtacagaccagacacggcggcggcggcgggagaggggattccctgcgcccccggacctcagggccgctcagattcctggagaggaagccaagtgtccttctgccctcccccggtatcccatccaaggcgatcagtccagaactggctctcggaagcgctcgggcaaagactgcgaagaagaaaagacatctggcggaaacctgtgcgcctggggcggtggaactcggggaggagagggagggatcagacaggagagtggggactaccccctctgctcccaaattggggcagcttcctgggtttccgattttctcatttccgtgggtaaaaaaccctgcccccaccgggcttacgcaatttttttaaggggagaggagggaaaaatttgtggggggtacgaaaaggcggaaagaaacagtcatttcgtcacatgggcttggttttcagtcttataaaaaggaaggttctctcggttagcgaccaattgtcatacgacttgcagtgagcgtcaggagcacgtccaggaactcctcagcagcgcctccttcagctccacagccagacgccctcagacagcaaagcctacccccgcgccgcgccctgcccgccgctg

SEQ ID NO: 5 - DNA, 986 bp, unidentified
  source 1..986: mol_type = other DNA
atgagacatattatctgccacggaggtgttattaccgaagaaatggccgccagtcttttggaccagctgatcgaagaggtactggctgataatcttccacctcctagccattttgaaccacctacccttcacgaactgtatgatttagacgtgacggcccccgaagatcccaacgaggaggcggtttcgcagatttttcccgactctgtaatgttggcggtgcaggaagggattgacttactcacttttccgccggcgcccggttctccggagccgcctcacctttcccggcagcccgagcagccggagcagagagccttgggtccggtttctatgccaaaccttgtaccggaggtgatcgatcttacctgccacgaggctggctttccacccagtgacgacgaggatgaagagggtgaggagtttgtgttagattatgtggagcaccccgggcacggttgcaggtcttgtcattatcaccggaggaatacgggggacccagatattatgtgttcgctttgctatatgaggacctgtggcatgtttgtctacagtaagtgaaaattatgggcagtgggtgatagagtggtgggtttggtgtggtaattttttttttaatttttacagttttgtggtttaaagaattttgtattgtgatttttttaaaaggtcctgtgtctgaacctgagcctgagcccgagccagaaccggagcctgcaagacctacccgccgtcctaaaatggcgcctgctatcctgagacgcccgacatcacctgtgtctagagaatgcaatagtagtacggatagctgtgactccggtccttctaacacacctcctgagatacacccggtggtcccgctgtgccccattaaaccagttgccgtgagagttggtgggcgtcgccaggctgtggaatgtatcgaggacttgcttaacgagcctgggcaacctttggacttgagctgtaaacgccccaggccataa

SEQ ID NO: 6 - DNA, 1795 bp, unidentified
  source 1..1795: mol_type = other DNA
atggaggcttgggagtgtttggaagatttttctgctgtgcgtaacttgctggaacagagctctaacagtacctcttggttttggaggtttctgtggggctcatcccaggcaaagttagtctgcagaattaaggaggattacaagtgggaatttgaagagcttttgaaatcctgtggtgagctgtttgattctttgaatctgggtcaccaggcgcttttccaagagaaggtcatcaagactttggatttttccacaccggggcgcgctgcggctgctgttgcttttttgagttttataaaggataaatggagcgaagaaacccatctgagcggggggtacctgctggattttctggccatgcatctgtggagagcggttgtgagacacaagaatcgcctgctactgttgtcttccgtccgcccggcgataataccgacggaggagcagcagcagcagcaggaggaagccaggcggcggcggcaggagcagagcccatggaacccgagagccggcctggaccctcgggaatgaatgttgtacaggtggctgaactgtatccagaactgagacgcattttgacaattacagaggatgggcaggggctaaagggggtaaagagggagcggggggcttgtgaggctacagaggaggctaggaatctagcttttagcttaatgaccagacaccgtcctgagtgtattacttttcaacagatcaaggataattgcgctaatgagcttgatctgctggcgcagaagtattccatagagcagctgaccacttactggctgcagccaggggatgattttgaggaggctattagggtatatgcaaaggtggcacttaggccagattgcaagtacaagatcagcaaacttgtaaatatcaggaattgttgctacatttctgggaacggggccgaggtggagatagatacggaggatagggtggcctttagatgtagcatgataaatatgtggccgggggtgcttggcatggacggggtggttattatgaatgtaaggtttactggccccaattttagcggtacggttttcctggccaataccaaccttatcctacacggtgtaagcttctatgggtttaacaatacctgtgtggaagcctggaccgatgtaagggttcggggctgtgccttttactgctgctggaagggggtggtgtgtcgccccaaaagcagggcttcaattaagaaatgcctctttgaaaggtgtaccttgggtatcctgtctgagggtaactccagggtgcgccacaatgtggcctccgactgtggttgcttcatgctagtgaaaagcgtggctgtgattaagcataacatggtatgtggcaactgcgaggacagggcctctcagatgctgacctgctcggacggcaactgtcacctgctgaagaccattcacgtagccagccactctcgcaaggcctggccagtgtttgagcataacatactgacccgctgttccttgcatttgggtaacaggaggggggtgttcctaccttaccaatgcaatttgagtcacactaagatattgcttgagcccgagagcatgtccaaggtgaacctgaacggggtgtttgacatgaccatgaagatctggaaggtgctgaggtacgatgagacccgcaccaggtgcagaccctgcgagtgtggcggtaaacatattaggaaccagcctgtgatgctggatgtgaccgaggagctgaggcccgatcacttggtgctggcctgcacccgcgctgagtttggctctagcgatgaagatacagattg

SEQ ID NO: 7 - DNA, 2793 bp, unidentified
  source 1..2793: mol_type = other DNA
atggacaagttttggtggcacgcagcctggggactctgcctcgtgccgctgagcctggcgcagatcgatttgaatataacctgccgctttgcaggtgtattccacgtggagaaaaatggtcgctacagcatctctcggacggaggccgctgacctctgcaaggctttcaatagcaccttgcccacaatggcccagatggagaaagctctgagcatcggatttgagacctgcaggtatgggttcatagaagggcacgtggtgattccccggatccaccccaactccatctgtgcagcaaacaacacaggggtgtacatcctcacatccaacacctcccagtatgacacatattgcttcaatgcttcagctccacctgaagaagattgtacatcagtcacagacctgcccaatgcctttgatggaccaattaccataactattgttaaccgtgatggcacccgctatgtccagaaaggagaatacagaacgaatcctgaagacatctaccccagcaaccctactgatgatgacgtgagcagcggctcctccagtgaaaggagcagcacttcaggaggttacatcttttacaccttttctactgtacaccccatcccagacgaagacagtccctggatcaccgacagcacagacagaatccctgctaccagacactcacatgggagtcaagaaggtggagcaaacacaacctctggtcctataaggacaccccaaattatcctggactacagcttcgggggtggggccgggcgcgacatccccccgccgctgatcgaggaggcgtgcgagctgcccgagtgccaggaggacgcgggcaacaaggtctgcagcctgcagtgcaacaaccacgcgtgcggctgggacggcggtgactgctccctcaacttcaatgacccctggaagaactgcacgcagtctctgcagtgctggaagtacttcagtgacggccactgtgacagccagtgcaactcagccggctgcctcttcgacggctttgactgccagcgtgcggaaggccagtgcaaccccctgtacgaccagtactgcaaggaccacttcagcgacgggcactgcgaccagggctgcaacagcgcggagtgcgagtgggacgggctggactgtgcggagcatgtacccgagaggctggcggccggcacgctggtggtggtggtgctgatgccgccggagcagctgcgcaacagctccttccacttcctgcgggagctcagccgcgtgctgcacaccaacgtggtcttcaagcgtgacgcacacggccagcagatgatcttcccctactacggccgcgaggaggagctgcgcaagcaccccatcaagcgtgccgccgagggctgggccgcacctgacgccctgctgggccaggtgaaggcctcgctgctccctggtggcagcgagggtgggcggcggcggagggagctggaccccatggacgtccgcggctccatcgtctacctggagattgacaaccggcagtgtgtgcaggcctcctcgcagtgcttccagagtgccaccgacgtggccgcattcctgggagcgctcgcctcgctgggcagcctcaacatcccctacaagatcgaggccgtgcagagtgagaccgtggagccgcccccgccggcgcagctgcacttcatgtacgtggcggcggccgcctttgtgcttctgttcttcgtgggctgcggggtgctgctgtcccgcaagcgccggcggcagcatggccagctctggttcatcctggactacagcttcgggggtggggccgggcgcgacatccccccgccgctgatcgaggaggcgtgcgagctgcccgagtgccaggaggacgcgggcaacaaggtctgcagcctgcagtgcaacaaccacgcgtgcggctgggacggcggtgactgctccctcaacttcaatgacccctggaagaactgcacgcagtctctgcagtgctggaagtacttcagtgacggccactgtgacagccagtgcaactcagccggctgcctcttcgacggctttgactgccagcgtgcggaaggccagtgcaaccccctgtacgaccagtactgcaaggaccacttcagcgacgggcactgcgaccagggctgcaacagcgcggagtgcgagtgggacgggctggactgtgcggagcatgtacccgagaggctggcggccggcacgctggtggtggtggtgctgatgccgccggagcagctgcgcaacagctccttccacttcctgcgggagctcagccgcgtgctgcacaccaacgtggtcttcaagcgtgacgcacacggccagcagatgatcttcccctactacggccgcgaggaggagctgcgcaagcaccccatcaagcgtgccgccgagggctgggccgcacctgacgccctgctgggccaggtgaaggcctcgctgctccctggtggcagcgagggtgggcggcggcggagggagctggaccccatggacgtccgcggctccatcgtctacctggagattgacaaccggcagtgtgtgcaggcctcctcgcagtgcttccagagtgccaccgacgtggccgcattcctgggagcgctcgcctcgctgggcagcctcaacatcccctacaagatcgaggccgtgcagagtgagaccgtggagccgcccccgccggcgcagctgcacttcatgtacgtggcggcggccgcctttgtgcttctgttcttcgtgggctgcggggtgctgctgtcccgcaagcgccggcggcagcatggccagctctggttc

SEQ ID NO: 8 - DNA, 968 bp, unidentified
  source 1..968: mol_type = other DNA
atgaagcgcgcaagaccgtctgaagataccttcaaccccgtgtatccatatgacactgaaaccggtcctccaactgtgccttttcttactcctccctttgtatcccccaatgggtttcaagagagtccccctggagttcttactttaaaatgtttaaccccactaacaaccacaggcggatctctacagctaaaagtgggagggggacttacagtggatgacactgatggtaccttacaagaaaacatacgtgctacagcacccattactaaaaataatcactctgtagaactatccattggaaatggattagaaactcaaaacaataaactatgtgccaaattgggaaatgggttaaaatttaacaacggtgacatttgtataaaggatagtattaacaccttatggactggaataaaccctccacctaactgtcaaattgtggaaaacactaatacaaatgatggcaaacttactttagtattagtaaaaaacggagggcttgttaatggctacgtgtctctagttggtgtatcagacactgtgaaccaaatgttcacacaaaagacagcaaacatccaattaagattatattttgactcttctggaaatctattaactgatgaatcagacttaaaaattccacttaaaaataaatcttctacagcgaccagtgaaactgtagccagcagcaaagcctttatgccaagtactacagcttatcccttcaacaccactactagggatagtgaaaactacattcatggaatatgttactacatgactagttatgatagaagtctatttcccttgaacatttctataatgctaaacagccgtatgatttcttccaatgttgcctatgccatacaatttgaatggaatctaaatgcaagtgaatctccagaaagcaacatagctacgctgaccacatccccctttttcttttcttacattacagaagacga

SEQ ID NO: 9 - DNA, 720 bp, unidentified
  source 1..720: mol_type = other DNA
atggtgagcaagggcgccgagctgttcaccggcatcgtgcccatcctgatcgagctgaatggcgatgtgaatggccacaagttcagcgtgagcggcgagggcgagggcgatgccacctacggcaagctgaccctgaagttcatctgcaccaccggcaagctgcctgtgccctggcccaccctggtgaccaccctgagctacggcgtgcagtgcttctcacgctaccccgatcacatgaagcagcacgacttcttcaagagcgccatgcctgagggctacatccaggagcgcaccatcttcttcgaggatgacggcaactacaagtcgcgcgccgaggtgaagttcgagggcgataccctggtgaatcgcatcgagctgaccggcaccgatttcaaggaggatggcaacatcctgggcaataagatggagtacaactacaacgcccacaatgtgtacatcatgaccgacaaggccaagaatggcatcaaggtgaacttcaagatccgccacaacatcgaggatggcagcgtgcagctggccgaccactaccagcagaatacccccatcggcgatggccctgtgctgctgcccgataaccactacctgtccacccagagcgccctgtccaaggaccccaacgagaagcgcgatcacatgatctacttcggcttcgtgaccgccgccgccatcacccacggcatggatgagctgtacaagtga

SEQ ID NO: 10 - protein, 245 aa, Homo sapiens
MDKFWWHAAWGLCLVPLSLAQIDLNITCRFAGVFHVEKNGRYSISRTEAADLCKAFNSTLPTMAQMEKALSIGFETCRYGFIEGHVVIPRIHPNSICAANNTGVYILTSNTSQYDTYCFNASAPPEEDCTSVTDLPNAFDGPITITIVNRDGTRYVQKGEYRTNPEDIYPSNPTDDDVSSGSSSERSSTSGGYIFYTFSTVHPIPDEDSPWITDSTDRIPATRHSHGSQEGGANTTSGPIRTPQI

SEQ ID NO: 11 - protein, 343 aa, Homo sapiens
ILDYSFGGGAGRDIPPPLIEEACELPECQEDAGNKVCSLQCNNHACGWDGGDCSLNFNDPWKNCTQSLQCWKYFSDGHCDSQCNSAGCLFDGFDCQRAEGQCNPLYDQYCKDHFSDGHCDQGCNSAECEWDGLDCAEHVPERLAAGTLVVVVLMPPEQLRNSSFHFLRELSRVLHTNVVFKRDAHGQQMIFPYYGREEELRKHPIKRAAEGWAAPDALLGQVKASLLPGGSEGGRRRRELDPMDVRGSIVYLEIDNRQCVQASSQCFQSATDVAAFLGALASLGSLNIPYKIEAVQSETVEPPPPAQLHFMYVAAAAFVLLFFVGCGVLLSRKRRRQHGQLWF

SEQ ID NO: 12 - protein, 363 aa, Homo sapiens
MALGLQRARSTTELRKEKSRDAARSRRSQETEVLYQLAHTLPFARGVSAHLDKASIMRLTISYLRMHRLCAAGEWNQVGAGGEPLDACYLKALEGFVMVLTAEGDMAYLSENVSKHLGLSQLELIGHSIFDFIHPCDQEELQDALTPQQTLSRRKVEAPTERCFSLRMKSTLTSRGRTLNLKAATWKVLNCSGHMRAYKPPAQTSPAGSPDSEPPLQCLVLICEAIPHPGSLEPPLGRGAFLSRHSLDMKFTYCDDRIAEVAGYSPDDLIGCSAYEYIHALDSDAVSKSIHTCMYPISPGAKPAATWPPADTRTPQLPIPQDALPPHLNTSSLLPKPQGTVSFLAPSYPVPRSFSPHLPPWWP

SEQ ID NO: 13 - protein, 951 aa, unidentified
MDKFWWHAAWGLCLVPLSLAQIDLNITCRFAGVFHVEKNGRYSISRTEAADLCKAFNSTLPTMAQMEKALSIGFETCRYGFIEGHVVIPRIHPNSICAANNTGVYILTSNTSQYDTYCFNASAPPEEDCTSVTDLPNAFDGPITITIVNRDGTRYVQKGEYRTNPEDIYPSNPTDDDVSSGSSSERSSTSGGYIFYTFSTVHPIPDEDSPWITDSTDRIPATRHSHGSQEGGANTTSGPIRTPQIILDYSFGGGAGRDIPPPLIEEACELPECQEDAGNKVCSLQCNNHACGWDGGDCSLNFNDPWKNCTQSLQCWKYFSDGHCDSQCNSAGCLFDGFDCQRAEGQCNPLYDQYCKDHFSDGHCDQGCNSAECEWDGLDCAEHVPERLAAGTLVVVVLMPPEQLRNSSFHFLRELSRVLHTNVVFKRDAHGQQMIFPYYGREEELRKHPIKRAAEGWAAPDALLGQVKASLLPGGSEGGRRRRELDPMDVRGSIVYLEIDNRQCVQASSQCFQSATDVAAFLGALASLGSLNIPYKIEAVQSETVEPPPPAQLHFMYVAAAAFVLLFFVGCGVLLSRKRRRQHGQLWFMALGLQRARSTTELRKEKSRDAARSRRSQETEVLYQLAHTLPFARGVSAHLDKASIMRLTISYLRMHRLCAAGEWNQVGAGGEPLDACYLKALEGFVMVLTAEGDMAYLSENVSKHLGLSQLELIGHSIFDFIHPCDQEELQDALTPQQTLSRRKVEAPTERCFSLRMKSTLTSRGRTLNLKAATWKVLNCSGHMRAYKPPAQTSPAGSPDSEPPLQCLVLICEAIPHPGSLEPPLGRGAFLSRHSLDMKFTYCDDRIAEVAGYSPDDLIGCSAYEYIHALDSDAVSKSIHTCMYPISPGAKPAATWPPADTRTPQLPIPQDALPPHLNTSSLLPKPQGTVSFLAPSYPVPRSFSPHLPPWWP

SEQ ID NO: 14 - protein, 322 aa, unidentified
MKRARPSEDTFNPVYPYDTETGPPTVPFLTPPFVSPNGFQESPPGVLTLKCLTPLTTTGGSLQLKVGGGLTVDDTDGTLQENIRATAPITKNNHSVELSIGNGLETQNNKLCAKLGNGLKFNNGDICIKDSINTLWTGINPPPNCQIVENTNTNDGKLTLVLVKNGGLVNGYVSLVGVSDTVNQMFTQKTANIQLRLYFDSSGNLLTDESDLKIPLKNKSSTATSETVASSKAFMPSTTAYPFNTTTRDSENYIHGICYYMTSYDRSLFPLNISIMLNSRMISSNVAYAIQFEWNLNASESPESNIATLTTSPFFFSYITED

SEQ ID NO: 15 - protein, 239 aa, unidentified
MVSKGAELFTGIVPILIELNGDVNGHKFSVSGEGEGDATYGKLTLKFICTTGKLPVPWPTLVTTLSYGVQCFSRYPDHMKQHDFFKSAMPEGYIQERTIFFEDDGNYKSRAEVKFEGDTLVNRIELTGTDFKEDGNILGNKMEYNYNAHNVYIMTDKAKNGIKVNFKIRHNIEDGSVQLADHYQQNTPIGDGPVLLPDNHYLSTQSALSKDPNEKRDHMIYFGFVTAAAITHGMDELYK

SEQ ID NO: 16 - DNA, 35 bp, synthetic construct
  source 1..35: mol_type = other DNA
agcggccgctgtcgattgaggtacctggtgtagtt

SEQ ID NO: 17 - DNA, 33 bp, synthetic construct
  source 1..33: mol_type = other DNA
tagtgatatcgaattacagcggcgggcagggcg

SEQ ID NO: 18 - DNA, 19 bp, synthetic construct
  source 1..19: mol_type = other DNA
ctagttgagcgggacaggg

SEQ ID NO: 19 - DNA, 18 bp, synthetic construct
  source 1..18: mol_type = other DNA
agagctgggaggagggca

SEQ ID NO: 20 - DNA, 24 bp, synthetic construct
  source 1..24: mol_type = other DNA
ggaataacctcttgcagtagtttc

SEQ ID NO: 21 - DNA, 18 bp, synthetic construct
  source 1..18: mol_type = other DNA
gccggtcatccccaaaag

SEQ ID NO: 22 - DNA, 19 bp, synthetic construct
  source 1..19: mol_type = other DNA
tcgcaacacgtaacgcaat

SEQ ID NO: 23 - DNA, 23 bp, synthetic construct
  source 1..23: mol_type = other DNA
acttctctttttccaccccattt

SEQ ID NO: 24 - DNA, 25 bp, synthetic construct
  source 1..25: mol_type = other DNA
aacaagtacgactcatggatttcct

SEQ ID NO: 25 - DNA, 16 bp, synthetic construct
  source 1..16: mol_type = other DNA
gcccgctccacgttga

SEQ ID NO: 26 - DNA, 26 bp, synthetic construct
  source 1..26: mol_type = other DNA
gatactcaggcagagatgatctaccc

SEQ ID NO: 27 - DNA, 22 bp, synthetic construct
  source 1..22: mol_type = other DNA
agaccaggcaccagaccaaaga

SEQ ID NO: 28 - DNA, 20 bp, synthetic construct
  source 1..20: mol_type = other DNA
gggagacatggcttacctgt

SEQ ID NO: 29 - DNA, 20 bp, synthetic construct
  source 1..20: mol_type = other DNA
gcgtactcttcatgcgcaag

SEQ ID NO: 30 - DNA, 20 bp, synthetic construct
  source 1..20: mol_type = other DNA
tacctccaccatgccaagtg

SEQ ID NO: 31 - DNA, 21 bp, synthetic construct
  source 1..21: mol_type = other DNA
atgattctgccctcctccttc

SEQ ID NO: 32 - DNA, 22 bp, synthetic construct
  source 1..22: mol_type = other DNA
aagatctcagtgcagaggctcg

SEQ ID NO: 33 - DNA, 21 bp, synthetic construct
  source 1..21: mol_type = other DNA
ttgcttgtccaggtggtccat

SEQ ID NO: 34 - DNA, 20 bp, synthetic construct
  source 1..20: mol_type = other DNA
gacagttacgcgcacatgaa

SEQ ID NO: 35 - DNA, 20 bp, synthetic construct
  source 1..20: mol_type = other DNA
taggtctgcgagctggtcat

SEQ ID NO: 36 - DNA, 25 bp, synthetic construct
  source 1..25: mol_type = other DNA
gccagcttcggagagttctgggatt

SEQ ID NO: 37 - DNA, 26 bp, synthetic construct
  source 1..26: mol_type = other DNA
cgggcacgaagtgcaatggtctttaa

SEQ ID NO: 38 - DNA, 22 bp, synthetic construct
  source 1..22: mol_type = other DNA
ttgtggttcttgcagatatggc

SEQ ID NO: 39 - DNA, 16 bp, synthetic construct
  source 1..16: mol_type = other DNA
tcggaatcccggcacc

SEQ ID NO: 40 - DNA, 18 bp, synthetic construct
  source 1..18: mol_type = other DNA
aaagcttcagcaggccac

SEQ ID NO: 41 - DNA, 21 bp, synthetic construct
  source 1..21: mol_type = other DNA
tttggtcctgtttcaagttcc

SEQ ID NO: 42 - DNA, 20 bp, synthetic construct
  source 1..20: mol_type = other DNA
ggtattcagccaaacgacca

SEQ ID NO: 43 - DNA, 20 bp, synthetic construct
  source 1..20: mol_type = other DNA
cacactcggaccacatcctt

SEQ ID NO: 44 - DNA, 20 bp, synthetic construct
  source 1..20: mol_type = other DNA
gtgatttgtgggcctgaaga

SEQ ID NO: 45 - DNA, 20 bp, synthetic construct
  source 1..20: mol_type = other DNA
acacagctgggtggaagaga

SEQ ID NO: 46 - DNA, 21 bp, synthetic construct
  source 1..21: mol_type = other DNA
tcctgcggatatttccagagg

SEQ ID NO: 47 - DNA, 22 bp, synthetic construct
  source 1..22: mol_type = other DNA
ggttcctacgatctgaccagaa

SEQ ID NO: 48 - DNA, 19 bp, synthetic construct
  source 1..19: mol_type = other DNA
ccagggtagctgctggagc

SEQ ID NO: 49 - DNA, 16 bp, synthetic construct
  source 1..16: mol_type = other DNA
tggcatggcgggttgt

SEQ ID NO: 50 - DNA, 23 bp, synthetic construct
  source 1..23: mol_type = other DNA
gctgaaagcttgcaactgccgac

SEQ ID NO: 51 - DNA, 23 bp, synthetic construct
  source 1..23: mol_type = other DNA
ggtatcgttggcagctcaggaac